European Patent Application EP 4 166 675 A1, published April 19, 2023. Title: Translation system with altered genetic code table. Applicant: CHUGAI SEIYAKU KABUSHIKI KAISHA. The sequence listing filed with the application follows.

SEQUENCE LISTING (283 sequences)

SEQ ID NO: 1 - DNA, 95 bp, Artificial Sequence
  D-1
ggcgtaatacgactcactatagtccccttcgtctagaggcccaggacaccgccctaagacggcggtaacaggggttcgaatcccctaggggacgc

SEQ ID NO: 2 - DNA, 95 bp, Artificial Sequence
  D-2
ggcgtaatacgactcactatagtccccttcgtctagaggcccaggacaccgcccttagacggcggtaacaggggttcgaatcccctaggggacgc

SEQ ID NO: 3 - DNA, 95 bp, Artificial Sequence
  D-3
ggcgtaatacgactcactatagtccccttcgtctagaggcccaggacaccgccctcagacggcggtaacaggggttcgaatcccctaggggacgc

SEQ ID NO: 4 - DNA, 95 bp, Artificial Sequence
  D-4
ggcgtaatacgactcactatagtccccttcgtctagaggcccaggacaccgccctaacacggcggtaacaggggttcgaatcccctaggggacgc

SEQ ID NO: 5 - DNA, 95 bp, Artificial Sequence
  D-5
ggcgtaatacgactcactatagtccccttcgtctagaggcccaggacaccgcccttacacggcggtaacaggggttcgaatcccctaggggacgc

SEQ ID NO: 6 - DNA, 95 bp, Artificial Sequence
  D-6
ggcgtaatacgactcactatagtccccttcgtctagaggcccaggacaccgccctcacacggcggtaacaggggttcgaatcccctaggggacgc

SEQ ID NO: 7 - DNA, 95 bp, Artificial Sequence
  D-7
ggcgtaatacgactcactatagtccccttcgtctagaggcccaggacaccgccctatgacggcggtaacaggggttcgaatcccctaggggacgc

SEQ ID NO: 8 - DNA, 95 bp, Artificial Sequence
  D-8
ggcgtaatacgactcactatagtccccttcgtctagaggcccaggacaccgccctttgacggcggtaacaggggttcgaatcccctaggggacgc

SEQ ID NO: 9 - DNA, 95 bp, Artificial Sequence
  D-9
ggcgtaatacgactcactatagtccccttcgtctagaggcccaggacaccgccctctgacggcggtaacaggggttcgaatcccctaggggacgc

SEQ ID NO: 10 - DNA, 95 bp, Artificial Sequence
  D-10
ggcgtaatacgactcactatagtccccttcgtctagaggcccaggacaccgccctattacggcggtaacaggggttcgaatcccctaggggacgc

SEQ ID NO: 11 - DNA, 95 bp, Artificial Sequence
  D-11
ggcgtaatacgactcactatagtccccttcgtctagaggcccaggacaccgcccttttacggcggtaacaggggttcgaatcccctaggggacgc

SEQ ID NO: 12 - DNA, 95 bp, Artificial Sequence
  D-12
ggcgtaatacgactcactatagtccccttcgtctagaggcccaggacaccgccctcttacggcggtaacaggggttcgaatcccctaggggacgc

SEQ ID NO: 13 - DNA, 95 bp, Artificial Sequence
  D-13
ggcgtaatacgactcactatagtccccttcgtctagaggcccaggacaccgccctatcacggcggtaacaggggttcgaatcccctaggggacgc

SEQ ID NO: 14 - DNA, 95 bp, Artificial Sequence
  D-14
ggcgtaatacgactcactatagtccccttcgtctagaggcccaggacaccgccctttcacggcggtaacaggggttcgaatcccctaggggacgc

SEQ ID NO: 15 - DNA, 95 bp, Artificial Sequence
  D-15
ggcgtaatacgactcactatagtccccttcgtctagaggcccaggacaccgccctctcacggcggtaacaggggttcgaatcccctaggggacgc

SEQ ID NO: 16 - DNA, 95 bp, Artificial Sequence
  D-16
ggcgtaatacgactcactatagtccccttcgtctagaggcccaggacaccgccctaaaacggcggtaacaggggttcgaatcccctaggggacgc

SEQ ID NO: 17 - DNA, 95 bp, Artificial Sequence
  D-17
ggcgtaatacgactcactatagtccccttcgtctagaggcccaggacaccgcccttaaacggcggtaacaggggttcgaatcccctaggggacgc

SEQ ID NO: 18 - DNA, 95 bp, Artificial Sequence
  D-18
ggcgtaatacgactcactatagtccccttcgtctagaggcccaggacaccgccctcaaacggcggtaacaggggttcgaatcccctaggggacgc

SEQ ID NO: 19 - DNA, 95 bp, Artificial Sequence
  D-19
ggcgtaatacgactcactatagtccccttcgtctagaggcccaggacaccgccctactacggcggtaacaggggttcgaatcccctaggggacgc

SEQ ID NO: 20 - DNA, 95 bp, Artificial Sequence
  D-20
ggcgtaatacgactcactatagtccccttcgtctagaggcccaggacaccgcccttctacggcggtaacaggggttcgaatcccctaggggacgc

SEQ ID NO: 21 - DNA, 95 bp, Artificial Sequence
  D-21
ggcgtaatacgactcactatagtccccttcgtctagaggcccaggacaccgccctcctacggcggtaacaggggttcgaatcccctaggggacgc

SEQ ID NO: 22 - DNA, 95 bp, Artificial Sequence
  D-22
ggcgtaatacgactcactatagtccccttcgtctagaggcccaggacaccgccctgcaacggcggtaacaggggttcgaatcccctaggggacgc

SEQ ID NO: 23 - DNA, 95 bp, Artificial Sequence
  D-23
ggcgtaatacgactcactatagtccccttcgtctagaggcccaggacaccgcccttcaacggcggtaacaggggttcgaatcccctaggggacgc

SEQ ID NO: 24 - DNA, 95 bp, Artificial Sequence
  D-24
ggcgtaatacgactcactatagtccccttcgtctagaggcccaggacaccgccctccaacggcggtaacaggggttcgaatcccctaggggacgc

SEQ ID NO: 25 - DNA, 95 bp, Artificial Sequence
  D-25
ggcgtaatacgactcactataggcggggtggagcagcctggtagctcgtcgggctcataacccgaagatcgtcggttcaaatccggcccccgcaa

SEQ ID NO: 26 - DNA, 95 bp, Artificial Sequence
  D-26
ggcgtaatacgactcactatagtccccttcgtctagaggcccaggacaccgccctgtgacggcggtaacaggggttcgaatcccctaggggacgc

SEQ ID NO: 27 - DNA, 95 bp, Artificial Sequence
  D-27
ggcgtaatacgactcactatagtccccttcgtctagaggcccaggacaccgccctgttacggcggtaacaggggttcgaatcccctaggggacgc

SEQ ID NO: 28 - DNA, 95 bp, Artificial Sequence
  D-28
ggcgtaatacgactcactatagtccccttcgtctagaggcccaggacaccgccctgtcacggcggtaacaggggttcgaatcccctaggggacgc

SEQ ID NO: 29 - DNA, 95 bp, Artificial Sequence
  D-29
ggcgtaatacgactcactatagtccccttcgtctagaggcccaggacaccgccctgaaacggcggtaacaggggttcgaatcccctaggggacgc

SEQ ID NO: 30 - DNA, 95 bp, Artificial Sequence
  D-30
ggcgtaatacgactcactatagtccccttcgtctagaggcccaggacaccgccctgctacggcggtaacaggggttcgaatcccctaggggacgc

SEQ ID NO: 31 - DNA, 95 bp, Artificial Sequence
  D-31
ggcgtaatacgactcactatagtccccttcgtctagaggcccaggacaccgcccttgaacggcggtaacaggggttcgaatcccctaggggacgc

SEQ ID NO: 32 - DNA, 95 bp, Artificial Sequence
  D-32
ggcgtaatacgactcactatagtccccttcgtctagaggcccaggacaccgcccttgtacggcggtaacaggggttcgaatcccctaggggacgc

SEQ ID NO: 33 - DNA, 95 bp, Artificial Sequence
  D-33
ggcgtaatacgactcactatagtccccttcgtctagaggcccaggacaccgcccttatacggcggtaacaggggttcgaatcccctaggggacgc

SEQ ID NO: 34 - DNA, 95 bp, Artificial Sequence
  D-34
ggcgtaatacgactcactataggccccttagctcagtggttagagcaggcgacttataatcgcttggtcgctggttcaagtccagcaggggccac

SEQ ID NO: 35 - DNA, 95 bp, Artificial Sequence
  D-76
ggcgtaatacgactcactatagtccccttcgtctagaggcccaggacaccgccctgcgacggcggtaacaggggttcgaatcccctaggggacgc

SEQ ID NO: 36 - DNA, 95 bp, Artificial Sequence
  D-77
ggcgtaatacgactcactatagtccccttcgtctagaggcccaggacaccgcccttcgacggcggtaacaggggttcgaatcccctaggggacgc

SEQ ID NO: 37 - DNA, 95 bp, Artificial Sequence
  D-78
ggcgtaatacgactcactatagtccccttcgtctagaggcccaggacaccgccctccgacggcggtaacaggggttcgaatcccctaggggacgc

SEQ ID NO: 38 - RNA, 74 nt, Artificial Sequence
  TR-1
guccccuucgucuagaggcccaggacaccgcccuaagacggcgguaacagggguucgaauccccuaggggacgc

SEQ ID NO: 39 - RNA, 74 nt, Artificial Sequence
  TR-2
guccccuucgucuagaggcccaggacaccgcccuuagacggcgguaacagggguucgaauccccuaggggacgc

SEQ ID NO: 40 - RNA, 74 nt, Artificial Sequence
  TR-3
guccccuucgucuagaggcccaggacaccgcccucagacggcgguaacagggguucgaauccccuaggggacgc

SEQ ID NO: 41 - RNA, 74 nt, Artificial Sequence
  TR-4
guccccuucgucuagaggcccaggacaccgcccuaacacggcgguaacagggguucgaauccccuaggggacgc

SEQ ID NO: 42 - RNA, 74 nt, Artificial Sequence
  TR-5
guccccuucgucuagaggcccaggacaccgcccuuacacggcgguaacagggguucgaauccccuaggggacgc

SEQ ID NO: 43 - RNA, 74 nt, Artificial Sequence
  TR-6
guccccuucgucuagaggcccaggacaccgcccucacacggcgguaacagggguucgaauccccuaggggacgc

SEQ ID NO: 44 - RNA, 74 nt, Artificial Sequence
  TR-7
guccccuucgucuagaggcccaggacaccgcccuaugacggcgguaacagggguucgaauccccuaggggacgc

SEQ ID NO: 45 - RNA, 74 nt, Artificial Sequence
  TR-8
guccccuucgucuagaggcccaggacaccgcccuuugacggcgguaacagggguucgaauccccuaggggacgc

SEQ ID NO: 46 - RNA, 74 nt, Artificial Sequence
  TR-9
guccccuucgucuagaggcccaggacaccgcccucugacggcgguaacagggguucgaauccccuaggggacgc

SEQ ID NO: 47 - RNA, 74 nt, Artificial Sequence
  TR-10
guccccuucgucuagaggcccaggacaccgcccuauuacggcgguaacagggguucgaauccccuaggggacgc

SEQ ID NO: 48 - RNA, 74 nt, Artificial Sequence
  TR-11
guccccuucgucuagaggcccaggacaccgcccuuuuacggcgguaacagggguucgaauccccuaggggacgc

SEQ ID NO: 49 - RNA, 74 nt, Artificial Sequence
  TR-12
guccccuucgucuagaggcccaggacaccgcccucuuacggcgguaacagggguucgaauccccuaggggacgc

SEQ ID NO: 50 - RNA, 74 nt, Artificial Sequence
  TR-13
guccccuucgucuagaggcccaggacaccgcccuaucacggcgguaacagggguucgaauccccuaggggacgc

SEQ ID NO: 51 - RNA, 74 nt, Artificial Sequence
  TR-14
guccccuucgucuagaggcccaggacaccgcccuuucacggcgguaacagggguucgaauccccuaggggacgc

SEQ ID NO: 52 - RNA, 74 nt, Artificial Sequence
  TR-15
guccccuucgucuagaggcccaggacaccgcccucucacggcgguaacagggguucgaauccccuaggggacgc

SEQ ID NO: 53 - RNA, 74 nt, Artificial Sequence
  TR-16
guccccuucgucuagaggcccaggacaccgcccuaaaacggcgguaacagggguucgaauccccuaggggacgc

SEQ ID NO: 54 - RNA, 74 nt, Artificial Sequence
  TR-17
guccccuucgucuagaggcccaggacaccgcccuuaaacggcgguaacagggguucgaauccccuaggggacgc

SEQ ID NO: 55 - RNA, 74 nt, Artificial Sequence
  TR-18
guccccuucgucuagaggcccaggacaccgcccucaaacggcgguaacagggguucgaauccccuaggggacgc

SEQ ID NO: 56 - RNA, 74 nt, Artificial Sequence
  TR-19
guccccuucgucuagaggcccaggacaccgcccuacuacggcgguaacagggguucgaauccccuaggggacgc

SEQ ID NO: 57 - RNA, 74 nt, Artificial Sequence
  TR-20
guccccuucgucuagaggcccaggacaccgcccuucuacggcgguaacagggguucgaauccccuaggggacgc

SEQ ID NO: 58 - RNA, 74 nt, Artificial Sequence
  TR-21
guccccuucgucuagaggcccaggacaccgcccuccuacggcgguaacagggguucgaauccccuaggggacgc

SEQ ID NO: 59 - RNA, 74 nt, Artificial Sequence
  TR-22
guccccuucgucuagaggcccaggacaccgcccugcaacggcgguaacagggguucgaauccccuaggggacgc

SEQ ID NO: 60 - RNA, 74 nt, Artificial Sequence
  TR-23
guccccuucgucuagaggcccaggacaccgcccuucaacggcgguaacagggguucgaauccccuaggggacgc

SEQ ID NO: 61 - RNA, 74 nt, Artificial Sequence
  TR-24
guccccuucgucuagaggcccaggacaccgcccuccaacggcgguaacagggguucgaauccccuaggggacgc

SEQ ID NO: 62 - RNA, 74 nt, Artificial Sequence
  TR-25
ggcgggguggagcagccugguagcucgucgggcucauaacccgaagaucgucgguucaaauccggcccccgcaa

SEQ ID NO: 63 - RNA, 74 nt, Artificial Sequence
  TR-26
guccccuucgucuagaggcccaggacaccgcccugugacggcgguaacagggguucgaauccccuaggggacgc

SEQ ID NO: 64 - RNA, 74 nt, Artificial Sequence
  TR-27
guccccuucgucuagaggcccaggacaccgcccuguuacggcgguaacagggguucgaauccccuaggggacgc

SEQ ID NO: 65 - RNA, 74 nt, Artificial Sequence
  TR-28
guccccuucgucuagaggcccaggacaccgcccugucacggcgguaacagggguucgaauccccuaggggacgc

SEQ ID NO: 66 - RNA, 74 nt, Artificial Sequence
  TR-29
guccccuucgucuagaggcccaggacaccgcccugaaacggcgguaacagggguucgaauccccuaggggacgc

SEQ ID NO: 67 - RNA, 74 nt, Artificial Sequence
  TR-30
guccccuucgucuagaggcccaggacaccgcccugcuacggcgguaacagggguucgaauccccuaggggacgc

SEQ ID NO: 68 - RNA, 74 nt, Artificial Sequence
  TR-31
guccccuucgucuagaggcccaggacaccgcccuugaacggcgguaacagggguucgaauccccuaggggacgc

SEQ ID NO: 69 - RNA, 74 nt, Artificial Sequence
  TR-32
guccccuucgucuagaggcccaggacaccgcccuuguacggcgguaacagggguucgaauccccuaggggacgc

SEQ ID NO: 70 - RNA, 74 nt, Artificial Sequence
  TR-33
guccccuucgucuagaggcccaggacaccgcccuuauacggcgguaacagggguucgaauccccuaggggacgc

SEQ ID NO: 71 - RNA, 74 nt, Artificial Sequence
  TR-34
ggccccuuagcucagugguuagagcaggcgacuuauaaucgcuuggucgcugguucaaguccagcaggggccac

SEQ ID NO: 72 - RNA, 74 nt, Artificial Sequence
  TR-35
guccccuucgucuagaggcccaggacaccgcccugcgacggcgguaacagggguucgaauccccuaggggacgc

SEQ ID NO: 73 - RNA, 74 nt, Artificial Sequence
  TR-36
guccccuucgucuagaggcccaggacaccgcccuucgacggcgguaacagggguucgaauccccuaggggacgc

SEQ ID NO: 74 - RNA, 74 nt, Artificial Sequence
  TR-37
guccccuucgucuagaggcccaggacaccgcccuccgacggcgguaacagggguucgaauccccuaggggacgc

SEQ ID NO: 75 - RNA, 76 nt, Artificial Sequence
  AAtR-1
guccccuucgucuagaggcccaggacaccgcccuaagacggcgguaacagggguucgaauccccuaggggacgcca

SEQ ID NO: 76 - RNA, 76 nt, Artificial Sequence
  AAtR-2
guccccuucgucuagaggcccaggacaccgcccuuagacggcgguaacagggguucgaauccccuaggggacgcca

SEQ ID NO: 77 - RNA, 76 nt, Artificial Sequence
  AAtR-3
guccccuucgucuagaggcccaggacaccgcccucagacggcgguaacagggguucgaauccccuaggggacgcca

SEQ ID NO: 78 - RNA, 76 nt, Artificial Sequence
  AAtR-4
guccccuucgucuagaggcccaggacaccgcccuaacacggcgguaacagggguucgaauccccuaggggacgcca

SEQ ID NO: 79 - RNA, 76 nt, Artificial Sequence
  AAtR-5
guccccuucgucuagaggcccaggacaccgcccuuacacggcgguaacagggguucgaauccccuaggggacgcca

SEQ ID NO: 80 - RNA, 76 nt, Artificial Sequence
  AAtR-6
guccccuucgucuagaggcccaggacaccgcccucacacggcgguaacagggguucgaauccccuaggggacgcca

SEQ ID NO: 81 - RNA, 76 nt, Artificial Sequence
  AAtR-7
guccccuucgucuagaggcccaggacaccgcccuaugacggcgguaacagggguucgaauccccuaggggacgcca

SEQ ID NO: 82 - RNA, 76 nt, Artificial Sequence
  AAtR-8
guccccuucgucuagaggcccaggacaccgcccuuugacggcgguaacagggguucgaauccccuaggggacgcca

SEQ ID NO: 83 - RNA, 76 nt, Artificial Sequence
  AAtR-9
guccccuucgucuagaggcccaggacaccgcccucugacggcgguaacagggguucgaauccccuaggggacgcca

SEQ ID NO: 84 - RNA, 76 nt, Artificial Sequence
  AAtR-10
guccccuucgucuagaggcccaggacaccgcccuauuacggcgguaacagggguucgaauccccuaggggacgcca

SEQ ID NO: 85 - RNA, 76 nt, Artificial Sequence
  AAtR-11
guccccuucgucuagaggcccaggacaccgcccuuuuacggcgguaacagggguucgaauccccuaggggacgcca

SEQ ID NO: 86 - RNA, 76 nt, Artificial Sequence
  AAtR-12
guccccuucgucuagaggcccaggacaccgcccucuuacggcgguaacagggguucgaauccccuaggggacgcca

SEQ ID NO: 87 - RNA, 76 nt, Artificial Sequence
  AAtR-13
guccccuucgucuagaggcccaggacaccgcccuaucacggcgguaacagggguucgaauccccuaggggacgcca

SEQ ID NO: 88 - RNA, 76 nt, Artificial Sequence
  AAtR-14
guccccuucgucuagaggcccaggacaccgcccuuucacggcgguaacagggguucgaauccccuaggggacgcca

SEQ ID NO: 89 - RNA, 76 nt, Artificial Sequence
  AAtR-15
guccccuucgucuagaggcccaggacaccgcccucucacggcgguaacagggguucgaauccccuaggggacgcca

SEQ ID NO: 90 - RNA, 76 nt, Artificial Sequence
  AAtR-16
guccccuucgucuagaggcccaggacaccgcccuaaaacggcgguaacagggguucgaauccccuaggggacgcca

SEQ ID NO: 91 - RNA, 76 nt, Artificial Sequence
  AAtR-17
guccccuucgucuagaggcccaggacaccgcccuuaaacggcgguaacagggguucgaauccccuaggggacgcca

SEQ ID NO: 92 - RNA, 76 nt, Artificial Sequence
  AAtR-18
guccccuucgucuagaggcccaggacaccgcccucaaacggcgguaacagggguucgaauccccuaggggacgcca

SEQ ID NO: 93 - RNA, 76 nt, Artificial Sequence
  AAtR-19
guccccuucgucuagaggcccaggacaccgcccuacuacggcgguaacagggguucgaauccccuaggggacgcca

SEQ ID NO: 94 - RNA, 76 nt, Artificial Sequence
  AAtR-20
guccccuucgucuagaggcccaggacaccgcccuucuacggcgguaacagggguucgaauccccuaggggacgcca

SEQ ID NO: 95 - RNA, 76 nt, Artificial Sequence
  AAtR-21
guccccuucgucuagaggcccaggacaccgcccuccuacggcgguaacagggguucgaauccccuaggggacgcca

SEQ ID NO: 96 - RNA, 76 nt, Artificial Sequence
  AAtR-22
guccccuucgucuagaggcccaggacaccgcccugcaacggcgguaacagggguucgaauccccuaggggacgcca

SEQ ID NO: 97 - RNA, 76 nt, Artificial Sequence
  AAtR-23
guccccuucgucuagaggcccaggacaccgcccuucaacggcgguaacagggguucgaauccccuaggggacgcca

SEQ ID NO: 98 - RNA, 76 nt, Artificial Sequence
  AAtR-24
guccccuucgucuagaggcccaggacaccgcccuccaacggcgguaacagggguucgaauccccuaggggacgcca

SEQ ID NO: 99 - RNA, 76 nt, Artificial Sequence
  AAtR-25
ggcgggguggagcagccugguagcucgucgggcucauaacccgaagaucgucgguucaaauccggcccccgcaaca

SEQ ID NO: 100 - RNA, 76 nt, Artificial Sequence
  AAtR-26
guccccuucgucuagaggcccaggacaccgcccugugacggcgguaacagggguucgaauccccuaggggacgcca

SEQ ID NO: 101 - RNA, 76 nt, Artificial Sequence
  AAtR-27
guccccuucgucuagaggcccaggacaccgcccuguuacggcgguaacagggguucgaauccccuaggggacgcca

SEQ ID NO: 102 - RNA, 76 nt, Artificial Sequence
  AAtR-28
guccccuucgucuagaggcccaggacaccgcccugcuacggcgguaacagggguucgaauccccuaggggacgcca

SEQ ID NO: 103 - RNA, 76 nt, Artificial Sequence; identical to SEQ ID NO: 81
  AAtR-29

SEQ ID NO: 104 - RNA, 76 nt, Artificial Sequence; identical to SEQ ID NO: 82
  AAtR-30

SEQ ID NO: 105 - RNA, 76 nt, Artificial Sequence; identical to SEQ ID NO: 83
  AAtR-31

SEQ ID NO: 106 - RNA, 76 nt, Artificial Sequence; identical to SEQ ID NO: 84
  AAtR-32

SEQ ID NO: 107 - RNA, 76 nt, Artificial Sequence; identical to SEQ ID NO: 85
  AAtR-33

SEQ ID NO: 108 - RNA, 76 nt, Artificial Sequence; identical to SEQ ID NO: 86
  AAtR-34

SEQ ID NO: 109 - RNA, 76 nt, Artificial Sequence; identical to SEQ ID NO: 87
  AAtR-35

SEQ ID NO: 110 - RNA, 76 nt, Artificial Sequence; identical to SEQ ID NO: 88
  AAtR-36

SEQ ID NO: 111 - RNA, 76 nt, Artificial Sequence; identical to SEQ ID NO: 89
  AAtR-37

SEQ ID NO: 112 - RNA, 76 nt, Artificial Sequence; identical to SEQ ID NO: 90
  AAtR-38

SEQ ID NO: 113 - RNA, 76 nt, Artificial Sequence; identical to SEQ ID NO: 91
  AAtR-39

SEQ ID NO: 114 - RNA, 76 nt, Artificial Sequence; identical to SEQ ID NO: 92
  AAtR-40

SEQ ID NO: 115 - RNA, 76 nt, Artificial Sequence; identical to SEQ ID NO: 93
  AAtR-41

SEQ ID NO: 116 - RNA, 76 nt, Artificial Sequence; identical to SEQ ID NO: 94
  AAtR-42

SEQ ID NO: 117 - RNA, 76 nt, Artificial Sequence; identical to SEQ ID NO: 95
  AAtR-43

SEQ ID NO: 118 - RNA, 76 nt, Artificial Sequence; identical to SEQ ID NO: 96
  AAtR-44

SEQ ID NO: 119 - RNA, 76 nt, Artificial Sequence; identical to SEQ ID NO: 97
  AAtR-45

SEQ ID NO: 120 - RNA, 76 nt, Artificial Sequence; identical to SEQ ID NO: 98
  AAtR-46

SEQ ID NO: 121 - RNA, 76 nt, Artificial Sequence; identical to SEQ ID NO: 100
  AAtR-47

SEQ ID NO: 122 - RNA, 76 nt, Artificial Sequence; identical to SEQ ID NO: 101
  AAtR-48

SEQ ID NO: 123 - RNA, 76 nt, Artificial Sequence
  AAtR-49
guccccuucgucuagaggcccaggacaccgcccugucacggcgguaacagggguucgaauccccuaggggacgcca

SEQ ID NO: 124 - RNA, 76 nt, Artificial Sequence
  AAtR-50
guccccuucgucuagaggcccaggacaccgcccugaaacggcgguaacagggguucgaauccccuaggggacgcca

SEQ ID NO: 125 - RNA, 76 nt, Artificial Sequence; identical to SEQ ID NO: 102
  AAtR-51

SEQ ID NO: 126 - RNA, 76 nt, Artificial Sequence
  AAtR-52
guccccuucgucuagaggcccaggacaccgcccuugaacggcgguaacagggguucgaauccccuaggggacgcca

SEQ ID NO: 127 - RNA, 76 nt, Artificial Sequence
  AAtR-53
guccccuucgucuagaggcccaggacaccgcccuuguacggcgguaacagggguucgaauccccuaggggacgcca

SEQ ID NO: 128 - RNA, 76 nt, Artificial Sequence
  AAtR-54
guccccuucgucuagaggcccaggacaccgcccuuauacggcgguaacagggguucgaauccccuaggggacgcca

SEQ ID NO: 129 - RNA, 76 nt, Artificial Sequence
  AAtR-55
ggccccuuagcucagugguuagagcaggcgacuuauaaucgcuuggucgcugguucaaguccagcaggggccacca

SEQ ID NO: 130 - RNA, 76 nt, Artificial Sequence; identical to SEQ ID NO: 129
  AAtR-56

SEQ ID NO: 131 - RNA, 76 nt, Artificial Sequence
  AAtR-57
guccccuucgucuagaggcccaggacaccgcccugcgacggcgguaacagggguucgaauccccuaggggacgcca

SEQ ID NO: 132 - RNA, 76 nt, Artificial Sequence
  AAtR-58
guccccuucgucuagaggcccaggacaccgcccuucgacggcgguaacagggguucgaauccccuaggggacgcca

SEQ ID NO: 133 - RNA, 76 nt, Artificial Sequence
  AAtR-59
guccccuucgucuagaggcccaggacaccgcccuccgacggcgguaacagggguucgaauccccuaggggacgcca

SEQ ID NO: 134 - RNA, 76 nt, Artificial Sequence
  mR-1
ggguuaacuuuaagaaggagauauacauaugacuuuuauuauugguuuucuuauuauuccgauugguuaagcuucg

SEQ ID NO: 135 - RNA, 76 nt, Artificial Sequence
  mR-2
ggguuaacuuuaagaaggagauauacauaugacuuuuauuauugguuuucuaauuauuccgauugguuaagcuucg

SEQ ID NO: 136 - RNA, 76 nt, Artificial Sequence
  mR-3
ggguuaacuuuaagaaggagauauacauaugacuuuuauuauugguuuucugauuauuccgauugguuaagcuucg

SEQ ID NO: 137 - RNA, 76 nt, Artificial Sequence
  mR-4
ggguuaacuuuaagaaggagauauacauaugacuuuuauuauugguuuuguuauuauuccgauugguuaagcuucg

SEQ ID NO: 138 - RNA, 76 nt, Artificial Sequence
  mR-5
ggguuaacuuuaagaaggagauauacauaugacuuuuauuauugguuuuguaauuauuccgauugguuaagcuucg

SEQ ID NO: 139 - RNA, 76 nt, Artificial Sequence
  mR-6
ggguuaacuuuaagaaggagauauacauaugacuuuuauuauugguuuugugauuauuccgauugguuaagcuucg

SEQ ID NO: 140 - RNA, 76 nt, Artificial Sequence
  mR-7
ggguuaacuuuaagaaggagauauacauaugacuuuuauuauugguuuucauauuauuccgauugguuaagcuucg

SEQ ID NO: 141 - RNA, 76 nt, Artificial Sequence
  mR-8
ggguuaacuuuaagaaggagauauacauaugacuuuuauuauugguuuucaaauuauuccgauugguuaagcuucg

SEQ ID NO: 142 - RNA, 76 nt, Artificial Sequence
  mR-9
ggguuaacuuuaagaaggagauauacauaugacuuuuauuauugguuuucagauuauuccgauugguuaagcuucg

SEQ ID NO: 143 - RNA, 76 nt, Artificial Sequence
  mR-10
ggguuaacuuuaagaaggagauauacauaugacuuuuauuauugguuuuaauauuauuccgauugguuaagcuucg

SEQ ID NO: 144 - RNA, 76 nt, Artificial Sequence
  mR-11
ggguuaacuuuaagaaggagauauacauaugacuuuuauuauugguuuuaaaauuauuccgauugguuaagcuucg

SEQ ID NO: 145 - RNA, 76 nt, Artificial Sequence
  mR-12
ggguuaacuuuaagaaggagauauacauaugacuuuuauuauugguuuuaagauuauuccgauugguuaagcuucg

SEQ ID NO: 146 - RNA, 76 nt, Artificial Sequence
  mR-13
ggguuaacuuuaagaaggagauauacauaugacuuuuauuauugguuuugauauuauuccgauugguuaagcuucg

SEQ ID NO: 147 - RNA, 76 nt, Artificial Sequence
  mR-14
ggguuaacuuuaagaaggagauauacauaugacuuuuauuauugguuuugaaauuauuccgauugguuaagcuucg

SEQ ID NO: 148 - RNA, 76 nt, Artificial Sequence
  mR-15
ggguuaacuuuaagaaggagauauacauaugacuuuuauuauugguuuugagauuauuccgauugguuaagcuucg

SEQ ID NO: 149 - RNA, 76 nt, Artificial Sequence
  mR-16
ggguuaacuuuaagaaggagauauacauaugacuguuauuauugguguuuuuauuauuccgauugguuaagcuucg

SEQ ID NO: 150 - RNA, 76 nt, Artificial Sequence
  mR-17
ggguuaacuuuaagaaggagauauacauaugacuguuauuauugguguuuuaauuauuccgauugguuaagcuucg

SEQ ID NO: 151 - RNA, 76 nt, Artificial Sequence
  mR-18
ggguuaacuuuaagaaggagauauacauaugacuguuauuauugguguuuugauuauuccgauugguuaagcuucg

SEQ ID NO: 152 - RNA, 76 nt, Artificial Sequence
  mR-19
ggguuaacuuuaagaaggagauauacauaugacuuuuauuauugguuuuaguauuauuccgauugguuaagcuucg

SEQ ID NO: 153 - RNA, 76 nt, Artificial Sequence
  mR-20
ggguuaacuuuaagaaggagauauacauaugacuuuuauuauugguuuuagaauuauuccgauugguuaagcuucg

SEQ ID NO: 154 - RNA, 76 nt, Artificial Sequence
  mR-21
ggguuaacuuuaagaaggagauauacauaugacuuuuauuauugguuuuaggauuauuccgauugguuaagcuucg

SEQ ID NO: 155 - RNA, 76 nt, Artificial Sequence
  mR-22
ggguuaacuuuaagaaggagauauacauaugacuuuuauuauugguuuuugcauuauuccgauugguuaagcuucg

SEQ ID NO: 156 - RNA, 76 nt, Artificial Sequence
  mR-23
ggguuaacuuuaagaaggagauauacauaugacuuuuauuauugguuuuugaauuauuccgauugguuaagcuucg

SEQ ID NO: 157 - RNA, 76 nt, Artificial Sequence
  mR-24
ggguuaacuuuaagaaggagauauacauaugacuuuuauuauugguuuuuggauuauuccgauugguuaagcuucg

SEQ ID NO: 158 - RNA, 76 nt, Artificial Sequence
  mR-25
ggguuaacuuuaagaaggagauauacauaugacuuuuauuauugguuuucacauuauuccgauugguuaagcuucg

SEQ ID NO: 159 - RNA, 76 nt, Artificial Sequence
  mR-26
ggguuaacuuuaagaaggagauauacauaugacuuuuauuauugguuuuaacauuauuccgauugguuaagcuucg

SEQ ID NO: 160 - RNA, 76 nt, Artificial Sequence
  mR-27
ggguuaacuuuaagaaggagauauacauaugacuuuuauuauugguuuugacauuauuccgauugguuaagcuucg

SEQ ID NO: 161 - RNA, 76 nt, Artificial Sequence
  mR-28
ggguuaacuuuaagaaggagauauacauaugacuguuauuauugguguuuucauuauuccgauugguuaagcuucg

SEQ ID NO: 162 - RNA, 76 nt, Artificial Sequence
  mR-29
ggguuaacuuuaagaaggagauauacauaugacuuuuauuauugguuuuagcauuauuccgauugguuaagcuucg

SEQ ID NO: 163 - RNA, 76 nt, Artificial Sequence
  mR-30
ggguuaacuuuaagaaggagauauacauaugacuuuuauuauugguuuuucuauuauuccgauugguuaagcuucg

SEQ ID NO: 164 - RNA, 76 nt, Artificial Sequence
  mR-31
ggguuaacuuuaagaaggagauauacauaugacuuuuauuauugguuuuuccauuauuccgauugguuaagcuucg

SEQ ID NO: 165 - RNA, 76 nt, Artificial Sequence
  mR-32
ggguuaacuuuaagaaggagauauacauaugacuuuuauuauugguuuuucaauuauuccgauugguuaagcuucg

SEQ ID NO: 166 - RNA, 76 nt, Artificial Sequence
  mR-33
ggguuaacuuuaagaaggagauauacauaugacuuuuauuauugguuuuucgauuauuccgauugguuaagcuucg

SEQ ID NO: 167 - RNA, 76 nt, Artificial Sequence
  mR-34
ggguuaacuuuaauaaggagauauaaauaugccguuuauuauugguuuuacuauuauuccgauugguuaagcuucg

SEQ ID NO: 168 - RNA, 76 nt, Artificial Sequence
  mR-35
ggguuaacuuuaauaaggagauauaaauaugccguuuauuauugguuuuaccauuauuccgauugguuaagcuucg

SEQ ID NO: 169 - RNA, 76 nt, Artificial Sequence
  mR-36
ggguuaacuuuaauaaggagauauaaauaugccguuuauuauugguuuuacaauuauuccgauugguuaagcuucg

SEQ ID NO: 170 - RNA, 76 nt, Artificial Sequence
  mR-37
ggguuaacuuuaauaaggagauauaaauaugccguuuauuauugguuuuacgauuauuccgauugguuaagcuucg

SEQ ID NO: 171 - RNA, 76 nt, Artificial Sequence
  mR-38
ggguuaacuuuaagaaggagauauacauaugacuuuucuacuagguuuuauucuacuaccgcuagguuaagcuucg

SEQ ID NO: 172 - RNA, 76 nt, Artificial Sequence
  mR-39
ggguuaacuuuaagaaggagauauacauaugacuuuucuacuagguuuuauccuacuaccgcuagguuaagcuucg

SEQ ID NO: 173 - RNA, 76 nt, Artificial Sequence
  mR-40
ggguuaacuuuaagaaggagauauacauaugacuuuucuacuagguuuuauacuacuaccgcuagguuaagcuucg

SEQ ID NO: 174 - RNA, 76 nt, Artificial Sequence
  mR-41
ggguuaacuuuaagaaggagauauacauaugacuuuucuacuagguuuuaugcuacuaccgcuagguuaagcuucg

SEQ ID NO: 175 - DNA, 97 bp, Artificial Sequence
  D-35
ggcgtaatacgactcactatagggttaactttaagaaggagatatacatatgacttttattattggttttcttattattccgattggttaagcttcg

SEQ ID NO: 176 - DNA, 97 bp, Artificial Sequence
  D-36
ggcgtaatacgactcactatagggttaactttaagaaggagatatacatatgacttttattattggttttctaattattccgattggttaagcttcg

SEQ ID NO: 177 - DNA, 97 bp, Artificial Sequence
  D-37
ggcgtaatacgactcactatagggttaactttaagaaggagatatacatatgacttttattattggttttctgattattccgattggttaagcttcg

SEQ ID NO: 178 - DNA, 97 bp, Artificial Sequence
  D-38
ggcgtaatacgactcactatagggttaactttaagaaggagatatacatatgacttttattattggttttgttattattccgattggttaagcttcg

SEQ ID NO: 179 - DNA, 97 bp, Artificial Sequence
  D-39
ggcgtaatacgactcactatagggttaactttaagaaggagatatacatatgacttttattattggttttgtaattattccgattggttaagcttcg

SEQ ID NO: 180 - DNA, 97 bp, Artificial Sequence
  D-40
ggcgtaatacgactcactatagggttaactttaagaaggagatatacatatgacttttattattggttttgtgattattccgattggttaagcttcg

SEQ ID NO: 181 - DNA, 97 bp, Artificial Sequence
  D-41
ggcgtaatacgactcactatagggttaactttaagaaggagatatacatatgacttttattattggttttcatattattccgattggttaagcttcg

SEQ ID NO: 182 - DNA, 97 bp, Artificial Sequence
  D-42
ggcgtaatacgactcactatagggttaactttaagaaggagatatacatatgacttttattattggttttcaaattattccgattggttaagcttcg

SEQ ID NO: 183 - DNA, 97 bp, Artificial Sequence
  D-43
ggcgtaatacgactcactatagggttaactttaagaaggagatatacatatgacttttattattggttttcagattattccgattggttaagcttcg

SEQ ID NO: 184 - DNA, 97 bp, Artificial Sequence
  D-44
ggcgtaatacgactcactatagggttaactttaagaaggagatatacatatgacttttattattggttttaatattattccgattggttaagcttcg

SEQ ID NO: 185 - DNA, 97 bp, Artificial Sequence
  D-45
ggcgtaatacgactcactatagggttaactttaagaaggagatatacatatgacttttattattggttttaaaattattccgattggttaagcttcg

SEQ ID NO: 186 - DNA, 97 bp, Artificial Sequence
  D-46
ggcgtaatacgactcactatagggttaactttaagaaggagatatacatatgacttttattattggttttaagattattccgattggttaagcttcg

SEQ ID NO: 187 - DNA, 97 bp, Artificial Sequence
  D-47
ggcgtaatacgactcactatagggttaactttaagaaggagatatacatatgacttttattattggttttgatattattccgattggttaagcttcg

SEQ ID NO: 188 - DNA, 97 bp, Artificial Sequence
  D-48
ggcgtaatacgactcactatagggttaactttaagaaggagatatacatatgacttttattattggttttgaaattattccgattggttaagcttcg

SEQ ID NO: 189 - DNA, 97 bp, Artificial Sequence
  D-49
ggcgtaatacgactcactatagggttaactttaagaaggagatatacatatgacttttattattggttttgagattattccgattggttaagcttcg

SEQ ID NO: 190 - DNA, 97 bp, Artificial Sequence
  D-50
ggcgtaatacgactcactatagggttaactttaagaaggagatatacatatgactgttattattggtgtttttattattccgattggttaagcttcg

SEQ ID NO: 191 - DNA, 97 bp, Artificial Sequence
  D-51
ggcgtaatacgactcactatagggttaactttaagaaggagatatacatatgactgttattattggtgttttaattattccgattggttaagcttcg

SEQ ID NO: 192 - DNA, 97 bp, Artificial Sequence
  D-52
ggcgtaatacgactcactatagggttaactttaagaaggagatatacatatgactgttattattggtgttttgattattccgattggttaagcttcg

SEQ ID NO: 193 - DNA, 97 bp, Artificial Sequence
  D-53
ggcgtaatacgactcactatagggttaactttaagaaggagatatacatatgacttttattattggttttagtattattccgattggttaagcttcg

SEQ ID NO: 194 - DNA, 97 bp, Artificial Sequence
  D-54
ggcgtaatacgactcactatagggttaactttaagaaggagatatacatatgacttttattattggttttagaattattccgattggttaagcttcg

SEQ ID NO: 195 - DNA, 97 bp, Artificial Sequence
  D-55
ggcgtaatacgactcactatagggttaactttaagaaggagatatacatatgacttttattattggttttaggattattccgattggttaagcttcg

SEQ ID NO: 196 - DNA, 97 bp, Artificial Sequence
  D-56
ggcgtaatacgactcactatagggttaactttaagaaggagatatacatatgacttttattattggtttttgcattattccgattggttaagcttcg

SEQ ID NO: 197 - DNA, 97 bp, Artificial Sequence
  D-57
ggcgtaatacgactcactatagggttaactttaagaaggagatatacatatgacttttattattggtttttgaattattccgattggttaagcttcg

SEQ ID NO: 198 - DNA, 97 bp, Artificial Sequence
  D-58
ggcgtaatacgactcactatagggttaactttaagaaggagatatacatatgacttttattattggtttttggattattccgattggttaagcttcg

SEQ ID NO: 199 - DNA, 97 bp, Artificial Sequence
  D-59
ggcgtaatacgactcactatagggttaactttaagaaggagatatacatatgacttttattattggttttcacattattccgattggttaagcttcg

SEQ ID NO: 200 - DNA, 97 bp, Artificial Sequence
  D-60
ggcgtaatacgactcactatagggttaactttaagaaggagatatacatatgacttttattattggttttaacattattccgattggttaagcttcg

SEQ ID NO: 201 - DNA, 97 bp, Artificial Sequence
  D-61
ggcgtaatacgactcactatagggttaactttaagaaggagatatacatatgacttttattattggttttgacattattccgattggttaagcttcg

SEQ ID NO: 202 - DNA, 97 bp, Artificial Sequence
  D-62
ggcgtaatacgactcactatagggttaactttaagaaggagatatacatatgactgttattattggtgttttcattattccgattggttaagcttcg

SEQ ID NO: 203 - DNA, 97 bp, Artificial Sequence
  D-63
ggcgtaatacgactcactatagggttaactttaagaaggagatatacatatgacttttattattggttttagcattattccgattggttaagcttcg

SEQ ID NO: 204 - DNA, 97 bp, Artificial Sequence
  D-64
ggcgtaatacgactcactatagggttaactttaagaaggagatatacatatgacttttattattggtttttctattattccgattggttaagcttcg

SEQ ID NO: 205 - DNA, 97 bp, Artificial Sequence
  D-65
ggcgtaatacgactcactatagggttaactttaagaaggagatatacatatgacttttattattggtttttccattattccgattggttaagcttcg

SEQ ID NO: 206 - DNA, 97 bp, Artificial Sequence
  D-66
ggcgtaatacgactcactatagggttaactttaagaaggagatatacatatgacttttattattggtttttcaattattccgattggttaagcttcg

SEQ ID NO: 207 - DNA, 97 bp, Artificial Sequence
  D-67
ggcgtaatacgactcactatagggttaactttaagaaggagatatacatatgacttttattattggtttttcgattattccgattggttaagcttcg

SEQ ID NO: 208 - DNA, 97 bp, Artificial Sequence
  D-68
ggcgtaatacgactcactatagggttaactttaataaggagatataaatatgccgtttattattggttttactattattccgattggttaagcttcg

SEQ ID NO: 209 - DNA, 97 bp, Artificial Sequence
  D-69
ggcgtaatacgactcactatagggttaactttaataaggagatataaatatgccgtttattattggttttaccattattccgattggttaagcttcg

SEQ ID NO: 210 - DNA, 97 bp, Artificial Sequence
  D-70
ggcgtaatacgactcactatagggttaactttaataaggagatataaatatgccgtttattattggttttacaattattccgattggttaagcttcg

SEQ ID NO: 211 - DNA, 97 bp, Artificial Sequence
  D-71
ggcgtaatacgactcactatagggttaactttaataaggagatataaatatgccgtttattattggttttacgattattccgattggttaagcttcg

SEQ ID NO: 212 - DNA, 97 bp, Artificial Sequence
  D-72
ggcgtaatacgactcactatagggttaactttaagaaggagatatacatatgacttttctactaggttttattctactaccgctaggttaagcttcg

SEQ ID NO: 213 - DNA, 97 bp, Artificial Sequence
  D-73
ggcgtaatacgactcactatagggttaactttaagaaggagatatacatatgacttttctactaggttttatcctactaccgctaggttaagcttcg

SEQ ID NO: 214 - DNA, 97 bp, Artificial Sequence
  D-74
ggcgtaatacgactcactatagggttaactttaagaaggagatatacatatgacttttctactaggttttatactactaccgctaggttaagcttcg

SEQ ID NO: 215 - DNA, 97 bp, Artificial Sequence
  D-75
ggcgtaatacgactcactatagggttaactttaagaaggagatatacatatgacttttctactaggttttatgctactaccgctaggttaagcttcg

SEQ ID NO: 216 - DNA, 97 bp, Artificial Sequence
  D-79
ggcgtaatacgactcactatagggttaactttaagaaggagatatacatatgacttttattattggttttcgtattattccgattggttaagcttcg

SEQ ID NO: 217 - DNA, 97 bp, Artificial Sequence
  D-80
ggcgtaatacgactcactatagggttaactttaagaaggagatatacatatgacttttattattggttttcgaattattccgattggttaagcttcg

SEQ ID NO: 218 - DNA, 97 bp, Artificial Sequence
  D-81
ggcgtaatacgactcactatagggttaactttaagaaggagatatacatatgacttttattattggttttcggattattccgattggttaagcttcg

SEQ ID NO: 219 - RNA, 76 nt, Artificial Sequence
  mR-42
ggguuaacuuuaagaaggagauauacauaugacuuuuauuauugguuuucguauuauuccgauugguuaagcuucg

SEQ ID NO: 220 - RNA, 76 nt, Artificial Sequence
  mR-43
ggguuaacuuuaagaaggagauauacauaugacuuuuauuauugguuuucgaauuauuccgauugguuaagcuucg

SEQ ID NO: 221 - RNA, 76 nt, Artificial Sequence
  mR-44
ggguuaacuuuaagaaggagauauacauaugacuuuuauuauugguuuucggauuauuccgauugguuaagcuucg

SEQ ID NO: 222 - protein, 18 aa, Artificial Sequence
  LCT12
  misc_feature (1)..(1): Xaa = BdpFL
XFTIFPGFIITTGTGTGA

SEQ ID NO: 223 - protein, 14 aa, Artificial Sequence
  LCT67
  misc_feature (1)..(1): Xaa = BdpFL
XFTFIIGFIIIPIG

SEQ ID NO: 224 - DNA, 96 bp, Artificial Sequence
  D-82
ggcgtaatacgactcactataggagcggtagttcagtcggttagaatacctgcctaugacgcagggggtcgcgggttcgagtcccgtccgttccgc

SEQ ID NO: 225 - DNA, 96 bp, Artificial Sequence
  D-83
ggcgtaatacgactcactataggagcggtagttcagtcggttagaatacctgcttaugatgcagggggtcgcgggttcgagtcccgtccgttccgc

SEQ ID NO: 226 - DNA, 96 bp, Artificial Sequence
  D-84
ggcgtaatacgactcactataggagcggtagttcagtcggttagaatacctgcctgugacgcagggggtcgcgggttcgagtcccgtccgttccgc

SEQ ID NO: 227 - DNA, 96 bp, Artificial Sequence
  D-85
ggcgtaatacgactcactataggagcggtagttcagtcggttagaatacctgcttgugatgcagggggtcgcgggttcgagtcccgtccgttccgc

SEQ ID NO: 228 - DNA, 96 bp, Artificial Sequence
  D-86
ggcgtaatacgactcactataggagcggtagttcagtcggttagaatacctgcctuugacgcagggggtcgcgggttcgagtcccgtccgttccgc

SEQ ID NO: 229 - DNA, 96 bp, Artificial Sequence
  D-87
ggcgtaatacgactcactataggagcggtagttcagtcggttagaatacctgcttuugatgcagggggtcgcgggttcgagtcccgtccgttccgc

SEQ ID NO: 230 - DNA, 96 bp, Artificial Sequence
  D-88
ggcgtaatacgactcactataggagcggtagttcagtcggttagaatacctgcctcugacgcagggggtcgcgggttcgagtcccgtccgttccgc

SEQ ID NO: 231 - DNA, 96 bp, Artificial Sequence
  D-89
ggcgtaatacgactcactataggagcggtagttcagtcggttagaatacctgcttcugatgcagggggtcgcgggttcgagtcccgtccgttccgc

SEQ ID NO: 232 - DNA, 96 bp, Artificial Sequence
  D-90
ggcgtaatacgactcactataggagcggtagttcagtcggttagaatacctgcctaucacgcagggggtcgcgggttcgagtcccgtccgttccgc

SEQ ID NO: 233 - DNA, 96 bp, Artificial Sequence
  D-91
ggcgtaatacgactcactataggagcggtagttcagtcggttagaatacctgcctuucacgcagggggtcgcgggttcgagtcccgtccgttccgc

SEQ ID NO: 234 - DNA, 96 bp, Artificial Sequence
  D-92
ggcgtaatacgactcactataggagcggtagttcagtcggttagaatacctgcctcucacgcagggggtcgcgggttcgagtcccgtccgttccgc

SEQ ID NO: 235 - DNA, 95 bp, Artificial Sequence
  D-93
ggcgtaatacgactcactataggctctgtagttcagtcggtagaacggcggattatgattccgtatgtcactggttcgagtccagtcagagccgc

SEQ ID NO: 236 - DNA, 95 bp, Artificial Sequence
  D-94
ggcgtaatacgactcactataggctctgtagttcagtcggtagaacggcggattgtgattccgtatgtcactggttcgagtccagtcagagccgc

SEQ ID NO: 237 - DNA, 95 bp, Artificial Sequence
  D-95
ggcgtaatacgactcactataggctctgtagttcagtcggtagaacggcggattttgattccgtatgtcactggttcgagtccagtcagagccgc

SEQ ID NO: 238 - DNA, 95 bp, Artificial Sequence
  D-96
ggcgtaatacgactcactataggctctgtagttcagtcggtagaacggcggattctgattccgtatgtcactggttcgagtccagtcagagccgc

SEQ ID NO: 239 - DNA, 95 bp, Artificial Sequence
  D-97
ggcgtaatacgactcactataggctctgtagttcagtcggtagaacggcggactatcactccgtatgtcactggttcgagtccagtcagagccgc

SEQ ID NO: 240 - DNA, 95 bp, Artificial Sequence
  D-98
ggcgtaatacgactcactataggctctgtagttcagtcggtagaacggcggactttcactccgtatgtcactggttcgagtccagtcagagccgc

SEQ ID NO: 241 - DNA, 95 bp, Artificial Sequence
  D-99
ggcgtaatacgactcactataggctctgtagttcagtcggtagaacggcggactctcactccgtatgtcactggttcgagtccagtcagagccgc

SEQ ID NO: 242 - RNA, 75 nt, Artificial Sequence
  TR-38
ggagcgguaguucagucgguuagaauaccugccuaugacgcagggggucgcggguucgagucccguccguuccgc

SEQ ID NO: 243 - RNA, 75 nt, Artificial Sequence
  TR-39
ggagcgguaguucagucgguuagaauaccugcuuaugaugcagggggucgcggguucgagucccguccguuccgc

SEQ ID NO: 244 - RNA, 75 nt, Artificial Sequence
  TR-40
ggagcgguaguucagucgguuagaauaccugccugugacgcagggggucgcggguucgagucccguccguuccgc

SEQ ID NO: 245 - RNA, 75 nt, Artificial Sequence
  TR-41
ggagcgguaguucagucgguuagaauaccugcuugugaugcagggggucgcggguucgagucccguccguuccgc

SEQ ID NO: 246 - RNA, 75 nt, Artificial Sequence
  TR-42
ggagcgguaguucagucgguuagaauaccugccuuugacgcagggggucgcggguucgagucccguccguuccgc

SEQ ID NO: 247 - RNA, 75 nt, Artificial Sequence
  TR-43
ggagcgguaguucagucgguuagaauaccugcuuuugaugcagggggucgcggguucgagucccguccguuccgc

SEQ ID NO: 248 - RNA, 75 nt, Artificial Sequence
  TR-44
ggagcgguaguucagucgguuagaauaccugccucugacgcagggggucgcggguucgagucccguccguuccgc

SEQ ID NO: 249 - RNA, 75 nt, Artificial Sequence
  TR-45
ggagcgguaguucagucgguuagaauaccugcuucugaugcagggggucgcggguucgagucccguccguuccgc

SEQ ID NO: 250 - RNA, 75 nt, Artificial Sequence
  TR-46
ggagcgguaguucagucgguuagaauaccugccuaucacgcagggggucgcggguucgagucccguccguuccgc

SEQ ID NO: 251 - RNA, 75 nt, Artificial Sequence
  TR-47
ggagcgguaguucagucgguuagaauaccugccuuucacgcagggggucgcggguucgagucccguccguuccgc

SEQ ID NO: 252 - RNA, 75 nt, Artificial Sequence
  TR-48
ggagcgguaguucagucgguuagaauaccugccucucacgcagggggucgcggguucgagucccguccguuccgc

SEQ ID NO: 253 - RNA, 74 nt, Artificial Sequence
  TR-49
ggcucuguaguucagucgguagaacggcggauuaugauuccguaugucacugguucgaguccagucagagccgc

SEQ ID NO: 254 - RNA, 74 nt, Artificial Sequence
  TR-50
ggcucuguaguucagucgguagaacggcggauugugauuccguaugucacugguucgaguccagucagagccgc

SEQ ID NO: 255 - RNA, 74 nt, Artificial Sequence
  TR-51
ggcucuguaguucagucgguagaacggcggauuuugauuccguaugucacugguucgaguccagucagagccgc

SEQ ID NO: 256 - RNA, 74 nt, Artificial Sequence
  TR-52
ggcucuguaguucagucgguagaacggcggauucugauuccguaugucacugguucgaguccagucagagccgc

SEQ ID NO: 257 - RNA, 74 nt, Artificial Sequence
  TR-53
ggcucuguaguucagucgguagaacggcggacuaucacuccguaugucacugguucgaguccagucagagccgc

SEQ ID NO: 258 - RNA, 74 nt, Artificial Sequence
  TR-54
ggcucuguaguucagucgguagaacggcggacuuucacuccguaugucacugguucgaguccagucagagccgc

SEQ ID NO: 259 - RNA, 74 nt, Artificial Sequence
  TR-55
ggcucuguaguucagucgguagaacggcggacucucacuccguaugucacugguucgaguccagucagagccgc

SEQ ID NO: 260 - RNA, 77 nt, Artificial Sequence
  AAtR-60
ggagcgguaguucagucgguuagaauaccugccuaugacgcagggggucgcggguucgagucccguccguuccgcca

SEQ ID NO: 261 - RNA, 77 nt, Artificial Sequence
  AAtR-61
ggagcgguaguucagucgguuagaauaccugccuuugacgcagggggucgcggguucgagucccguccguuccgcca

SEQ ID NO: 262 - RNA, 77 nt, Artificial Sequence
  AAtR-62
ggagcgguaguucagucgguuagaauaccugccucugacgcagggggucgcggguucgagucccguccguuccgcca

SEQ ID NO: 263 - RNA, 77 nt, Artificial Sequence
  AAtR-63
ggagcgguaguucagucgguuagaauaccugcuuaugaugcagggggucgcggguucgagucccguccguuccgcca

SEQ ID NO: 264 - RNA, 77 nt, Artificial Sequence
  AAtR-64
ggagcgguaguucagucgguuagaauaccugcuuuugaugcagggggucgcggguucgagucccguccguuccgcca

SEQ ID NO: 265 - RNA, 77 nt, Artificial Sequence
  AAtR-65
ggagcgguaguucagucgguuagaauaccugcuucugaugcagggggucgcggguucgagucccguccguuccgcca

SEQ ID NO: 266 - RNA, 77 nt, Artificial Sequence
  AAtR-66
ggagcgguaguucagucgguuagaauaccugccugugacgcagggggucgcggguucgagucccguccguuccgcca

SEQ ID NO: 267 - RNA, 77 nt, Artificial Sequence; identical to SEQ ID NO: 261
  AAtR-67

SEQ ID NO: 268 - RNA, 77 nt, Artificial Sequence; identical to SEQ ID NO: 262
  AAtR-68

SEQ ID NO: 269 - RNA, 77 nt, Artificial Sequence
  AAtR-69
ggagcgguaguucagucgguuagaauaccugcuugugaugcagggggucgcggguucgagucccguccguuccgcca

SEQ ID NO: 270 - RNA, 77 nt, Artificial Sequence; identical to SEQ ID NO: 264
  AAtR-70

SEQ ID NO: 271 - RNA, 77 nt, Artificial Sequence; identical to SEQ ID NO: 265
  AAtR-71

SEQ ID NO: 272 - RNA, 77 nt, Artificial Sequence
  AAtR-72
ggagcgguaguucagucgguuagaauaccugccuaucacgcagggggucgcggguucgagucccguccguuccgcca

SEQ ID NO: 273 - RNA, 77 nt, Artificial Sequence
  AAtR-73
ggagcgguaguucagucgguuagaauaccugccuuucacgcagggggucgcggguucgagucccguccguuccgcca

SEQ ID NO: 274 - RNA, 77 nt, Artificial Sequence
  AAtR-74
ggagcgguaguucagucgguuagaauaccugccucucacgcagggggucgcggguucgagucccguccguuccgcca

SEQ ID NO: 275 - RNA, 76 nt, Artificial Sequence
  AAtR-75
ggcucuguaguucagucgguagaacggcggauuaugauuccguaugucacugguucgaguccagucagagccgcca

SEQ ID NO: 276 - RNA, 76 nt, Artificial Sequence
  AAtR-76
ggcucuguaguucagucgguagaacggcggauuuugauuccguaugucacugguucgaguccagucagagccgcca

SEQ ID NO: 277 - RNA, 76 nt, Artificial Sequence
  AAtR-77
ggcucuguaguucagucgguagaacggcggauucugauuccguaugucacugguucgaguccagucagagccgcca

SEQ ID NO: 278 - RNA, 76 nt, Artificial Sequence
  AAtR-78
ggcucuguaguucagucgguagaacggcggauugugauuccguaugucacugguucgaguccagucagagccgcca

SEQ ID NO: 279 - RNA, 76 nt, Artificial Sequence; identical to SEQ ID NO: 276
  AAtR-79

SEQ ID NO: 280 - RNA, 76 nt, Artificial Sequence; identical to SEQ ID NO: 277
  AAtR-80

SEQ ID NO: 281 - RNA, 76 nt, Artificial Sequence
  AAtR-81
ggcucuguaguucagucgguagaacggcggacuaucacuccguaugucacugguucgaguccagucagagccgcca

SEQ ID NO: 282 - RNA, 76 nt, Artificial Sequence
  AAtR-82
ggcucuguaguucagucgguagaacggcggacuuucacuccguaugucacugguucgaguccagucagagccgcca

SEQ ID NO: 283 - RNA, 76 nt, Artificial Sequence
  AAtR-83
ggcucuguaguucagucgguagaacggcggacucucacuccguaugucacugguucgaguccagucagagccgcca